European Patent Specification EP 2 879 701 B1, published November 15, 2023. Title: COMPOSITIONS AND METHODS FOR TREATING AN ACTIVE MYCOBACTERIUM TUBERCULOSIS INFECTION. Applicant: Infectious Disease Research Institute Reed, Steven G. Coler, Rhea N. The sequence listing filed with the application follows.

SEQUENCE LISTING (8 sequences)

SEQ ID NO: 1 - protein, 911 aa, Artificial Sequence
  Synthetic Construct
MGSSHHHHHHSSGLVPRGSHMTINYQFGDVDAHGAMIRAQAGSLEAEHQAIISDVLTASDFWGGAGSAACQGFITQLGRNFQVIYEQANAHGQKVQAAGNNMAQTDSAVGSSWAGTHLANGSMSEVMMSEIAGLPIPPIIHYGAIAYAPSGASGKAWHQRTPARAEQVALEKCGDKTCKVVSRFTRCGAVAYNGSKYQGGTGLTRRAAEDDAVNRLEGGRIVNWACNELMTSRFMTDPHAMRDMAGRFEVHAQTVEDEARRMWASAQNISGAGWSGMAEATSLDTMTQMNQAFRNIVNMLHGVRDGLVRDANNYEQQEQASQQILSSVDINFAVLPPEVNSARIFAGAGLGPMLAAASAWDGLAEELHAAAGSFASVTTGLAGDAWHGPASLAMTRAASPYVGWLNTAAGQAAQAAGQARLAASAFEATLAATVSPAMVAANRTRLASLVAANLLGQNAPAIAAAEAEYEQIWAQDVAAMFGYHSAASAVATQLAPIQEGLQQQLQNVLAQLASGNLGSGNVGVGNIGNDNIGNANIGFGNRGDANIGIGNIGDRNLGIGNTGNWNIGIGITGNGQIGFGKPANPDVLVVGNGGPGVTALVMGGTDSLLPLPNIPLLEYAARFITPVHPGYTATFLETPSQFFPFTGLNSLTYDVSVAQGVTNLHTAIMAQLAAGNEVVVFGTSQSATIATFEMRYLQSLPAHLRPGLDELSFTLTGNPNRPDGGILTRFGFSIPQLGFTLSGATPADAYPTVDYAFQYDGVNDFPKYPLNVFATANAIAGILFLHSGLIALPPDLASGVVQPVSSPDVLTTYILLPSQDLPLLVPLRAIPLLGNPLADLIQPDLRVLVELGYDRTAHQDVPSPFGLFPDVDWAEVAADLQQGAVQGVNDALSGLGLPPPWQPALPRLFST

SEQ ID NO: 2 - protein, 891 aa, Artificial Sequence
  Synthetic Construct
MTINYQFGDVDAHGAMIRAQAGSLEAEHQAIISDVLTASDFWGGAGSAACQGFITQLGRNFQVIYEQANAHGQKVQAAGNNMAQTDSAVGSSWAGTHLANGSMSEVMMSEIAGLPIPPIIHYGAIAYAPSGASGKAWHQRTPARAEQVALEKCGDKTCKVVSRFTRCGAVAYNGSKYQGGTGLTRRAAEDDAVNRLEGGRIVNWACNELMTSRFMTDPHAMRDMAGRFEVHAQTVEDEARRMWASAQNISGAGWSGMAEATSLDTMTQMNQAFRNIVNMLHGVRDGLVRDANNYEQQEQASQQILSSVDINFAVLPPEVNSARIFAGAGLGPMLAAASAWDGLAEELHAAAGSFASVTTGLAGDAWHGPASLAMTRAASPYVGWLNTAAGQAAQAAGQARLAASAFEATLAATVSPAMVAANRTRLASLVAANLLGQNAPAIAAAEAEYEQIWAQDVAAMFGYHSAASAVATQLAPIQEGLQQQLQNVLAQLASGNLGSGNVGVGNIGNDNIGNANIGFGNRGDANIGIGNIGDRNLGIGNTGNWNIGIGITGNGQIGFGKPANPDVLVVGNGGPGVTALVMGGTDSLLPLPNIPLLEYAARFITPVHPGYTATFLETPSQFFPFTGLNSLTYDVSVAQGVTNLHTAIMAQLAAGNEVVVFGTSQSATIATFEMRYLQSLPAHLRPGLDELSFTLTGNPNRPDGGILTRFGFSIPQLGFTLSGATPADAYPTVDYAFQYDGVNDFPKYPLNVFATANAIAGILFLHSGLIALPPDLASGVVQPVSSPDVLTTYILLPSQDLPLLVPLRAIPLLGNPLADLIQPDLRVLVELGYDRTAHQDVPSPFGLFPDVDWAEVAADLQQGAVQGVNDALSGLGLPPPWQPALPRLFST

SEQ ID NO: 3 - protein, 818 aa, Artificial Sequence
  Synthetic Construct
MGSSHHHHHHSSGLVPRGSHMGTHLANGSMSEVMMSEIAGLPIPPIIHYGAIAYAPSGASGKAWHQRTPARAEQVALEKCGDKTCKVVSRFTRCGAVAYNGSKYQGGTGLTRRAAEDDAVNRLEGGRIVNWACNELMTSRFMTDPHAMRDMAGRFEVHAQTVEDEARRMWASAQNISGAGWSGMAEATSLDTMTQMNQAFRNIVNMLHGVRDGLVRDANNYEQQEQASQQILSSVDINFAVLPPEVNSARIFAGAGLGPMLAAASAWDGLAEELHAAAGSFASVTTGLAGDAWHGPASLAMTRAASPYVGWLNTAAGQAAQAAGQARLAASAFEATLAATVSPAMVAANRTRLASLVAANLLGQNAPAIAAAEAEYEQIWAQDVAAMFGYHSAASAVATQLAPIQEGLQQQLQNVLAQLASGNLGSGNVGVGNIGNDNIGNANIGFGNRGDANIGIGNIGDRNLGIGNTGNWNIGIGITGNGQIGFGKPANPDVLVVGNGGPGVTALVMGGTDSLLPLPNIPLLEYAARFITPVHPGYTATFLETPSQFFPFTGLNSLTYDVSVAQGVTNLHTAIMAQLAAGNEVVVFGTSQSATIATFEMRYLQSLPAHLRPGLDELSFTLTGNPNRPDGGILTRFGFSIPQLGFTLSGATPADAYPTVDYAFQYDGVNDFPKYPLNVFATANAIAGILFLHSGLIALPPDLASGVVQPVSSPDVLTTYILLPSQDLPLLVPLRAIPLLGNPLADLIQPDLRVLVELGYDRTAHQDVPSPFGLFPDVDWAEVAADLQQGAVQGVNDALSGLGLPPPWQPALPRLFST

SEQ ID NO: 4 - protein, 795 aa, Artificial Sequence
  Synthetic Construct
HLANGSMSEVMMSEIAGLPIPPIIHYGAIAYAPSGASGKAWHQRTPARAEQVALEKCGDKTCKVVSRFTRCGAVAYNGSKYQGGTGLTRRAAEDDAVNRLEGGRIVNWACNELMTSRFMTDPHAMRDMAGRFEVHAQTVEDEARRMWASAQNISGAGWSGMAEATSLDTMTQMNQAFRNIVNMLHGVRDGLVRDANNYEQQEQASQQILSSVDINFAVLPPEVNSARIFAGAGLGPMLAAASAWDGLAEELHAAAGSFASVTTGLAGDAWHGPASLAMTRAASPYVGWLNTAAGQAAQAAGQARLAASAFEATLAATVSPAMVAANRTRLASLVAANLLGQNAPAIAAAEAEYEQIWAQDVAAMFGYHSAASAVATQLAPIQEGLQQQLQNVLAQLASGNLGSGNVGVGNIGNDNIGNANIGFGNRGDANIGIGNIGDRNLGIGNTGNWNIGIGITGNGQIGFGKPANPDVLVVGNGGPGVTALVMGGTDSLLPLPNIPLLEYAARFITPVHPGYTATFLETPSQFFPFTGLNSLTYDVSVAQGVTNLHTAIMAQLAAGNEVVVFGTSQSATIATFEMRYLQSLPAHLRPGLDELSFTLTGNPNRPDGGILTRFGFSIPQLGFTLSGATPADAYPTVDYAFQYDGVNDFPKYPLNVFATANAIAGILFLHSGLIALPPDLASGVVQPVSSPDVLTTYILLPSQDLPLLVPLRAIPLLGNPLADLIQPDLRVLVELGYDRTAHQDVPSPFGLFPDVDWAEVAADLQQGAVQGVNDALSGLGLPPPWQPALPRLFST

SEQ ID NO: 5 - protein, 143 aa, Mycobacterium tuberculosis
MITNLRRRTAMAAAGLGAALGLGILLVPTVDAHLANGSMSEVMMSEIAGLPIPPIIHYGAIAYAPSGASGKAWHQRTPARAEQVALEKCGDKTCKVVSRFTRCGAVAYNGSKYQGGTGLTRRAAEDDAVNRLEGGRIVNWACN

SEQ ID NO: 6 - protein, 98 aa, Mycobacterium tuberculosis
MTSRFMTDPHAMRDMAGRFEVHAQTVEDEARRMWASAQNISGAGWSGMAEATSLDTMTQMNQAFRNIVNMLHGVRDGLVRDANNYEQQEQASQQILSS

SEQ ID NO: 7 - protein, 580 aa, Mycobacterium tuberculosis
MNFAVLPPEVNSARIFAGAGLGPMLAAASAWDGLAEELHAAAGSFASVTTGLAGDAWHGPASLAMTRAASPYVGWLNTAAGQAAQAAGQARLAASAFEATLAATVSPAMVAANRTRLASLVAANLLGQNAPAIAAAEAEYEQIWAQDVAAMFGYHSAASAVATQLAPIQEGLQQQLQNVLAQLASGNLGSGNVGVGNIGNDNIGNANIGFGNRGDANIGIGNIGDRNLGIGNTGNWNIGIGITGNGQIGFGKPANPDVLVVGNGGPGVTALVMGGTDSLLPLPNIPLLEYAARFITPVHPGYTATFLETPSQFFPFTGLNSLTYDVSVAQGVTNLHTAIMAQLAAGNEVVVFGTSQSATIATFEMRYLQSLPAHLRPGLDELSFTLTGNPNRPDGGILTRFGFSIPQLGFTLSGATPADAYPTVDYAFQYDGVNDFPKYPLNVFATANAIAGILFLHSGLIALPPDLASGVVQPVSSPDVLTTYILLPSQDLPLLVPLRAIPLLGNPLADLIQPDLRVLVELGYDRTAHQDVPSPFGLFPDVDWAEVAADLQQGAVQGVNDALSGLGLPPPWQPALPRLF

SEQ ID NO: 8 - protein, 94 aa, Mycobacterium tuberculosis
MTINYQFGDVDAHGAMIRAQAGSLEAEHQAIISDVLTASDFWGGAGSAACQGFITQLGRNFQVIYEQANAHGQKVQAAGNNMAQTDSAVGSSWA